European Patent Specification EP 3 668 998 B1, published April 23, 2025. Title: Ligation probe. Applicant: CartaNA AB. The sequence listing filed with the application follows.

SEQUENCE LISTING (281 sequences)

SEQ ID NO: 1 - RNA, 41 nt, Homo sapiens
aacuugugguaguuggagcugguggcguaggcaagagugcc

SEQ ID NO: 2 - DNA, 70 bp, Artificial Sequence
  KRASwt_PLP
  misc_feature (1)..(1): 5' Phosphate
agctccaactaccacaaaaaaaaaaagtagccgtgactatcgactaaaaaaaaaacttgcctacgccacc

SEQ ID NO: 3 - RNA, 22 nt, Homo sapiens
ugagguaggagguuguauaguu

SEQ ID NO: 4 - RNA, 22 nt, Homo sapiens
agagguaguagguugcauaguu

SEQ ID NO: 5 - DNA, 65 bp, Artificial Sequence
  let7-a_PLP_1
  misc_feature (1)..(1): 5' Phosphate
ctactacctcaaaaaaaaaaacctcaatgcacatgtttggctccaaaaaaaaaaaactatacaac

SEQ ID NO: 6 - DNA, 65 bp, Artificial Sequence
  let7-f_PLP_1
  misc_feature (1)..(1): 5' Phosphate
ctactacctcaaaaaaaaaaacctcaatgcacatgtttggctccaaaaaaaaaaaactatacaat

SEQ ID NO: 7 - DNA, 65 bp, Artificial Sequence
  let7-e_PLP_1
  misc_feature (1)..(1): 5' Phosphate
ctcctacctcaaaaaaaaaaacctcaatgcacatgtttggctccaaaaaaaaaaaactatacaac

SEQ ID NO: 8 - DNA, 65 bp, Artificial Sequence
  let7-d_PLP_1
  misc_feature (1)..(1): 5' Phosphate
ctactacctctaaaaaaaaaacctcaatgcacatgtttggctccaaaaaaaaaaaactatgcaac

SEQ ID NO: 9 - DNA, 65 bp, Artificial Sequence; identical to SEQ ID NO: 5
  let7-a_PLP_RNA_1
  misc_feature (1)..(1): 5' Phosphate
  misc_feature (65)..(65): RNA

SEQ ID NO: 10 - DNA, 65 bp, Artificial Sequence
  let7-f_PLP_RNA_1
  misc_feature (1)..(1): 5' Phosphate
  misc_feature (65)..(65): RNA
ctactacctcaaaaaaaaaaacctcaatgcacatgtttggctccaaaaaaaaaaaactatacaau

SEQ ID NO: 11 - DNA, 65 bp, Artificial Sequence; identical to SEQ ID NO: 7
  let7-e_PLP_RNA_1
  misc_feature (1)..(1): 5' Phosphate
  misc_feature (65)..(65): RNA

SEQ ID NO: 12 - DNA, 65 bp, Artificial Sequence; identical to SEQ ID NO: 8
  let7-d_PLP_RNA_1
  misc_feature (1)..(1): 5' Phosphate
  misc_feature (65)..(65): RNA

SEQ ID NO: 13 - RNA, 25 nt, Artificial Sequence
  benchm_templ_C
ucucgcugucaucccuauauccucg

SEQ ID NO: 14 - RNA, 25 nt, Artificial Sequence
  benchm_templ_A
ucucgcugucauaccuauauccucg

SEQ ID NO: 15 - RNA, 25 nt, Artificial Sequence
  benchm_templ_G
ucucgcugucaugccuauauccucg

SEQ ID NO: 16 - RNA, 25 nt, Artificial Sequence
  benchm_templ_U
ucucgcugucauuccuauauccucg

SEQ ID NO: 17 - DNA, 65 bp, Artificial Sequence
  3'T_PLP_2
  misc_feature (1)..(1): 5' Phosphate
atgacagcgagaaaaaaaaaaaagtagccgtgactatcgactaaaaaaaaaacgaggatataggt

SEQ ID NO: 18 - DNA, 65 bp, Artificial Sequence
  3'G_PLP_2
  misc_feature (1)..(1): 5' Phosphate
atgacagcgagaaaaaaaaaaaagtagccgtgactatcgactaaaaaaaaaacgaggatataggg

SEQ ID NO: 19 - DNA, 65 bp, Artificial Sequence
  3'A_PLP_2
  misc_feature (1)..(1): 5' Phosphate
atgacagcgagaaaaaaaaaaaagtagccgtgactatcgactaaaaaaaaaacgaggatatagga

SEQ ID NO: 20 - DNA, 65 bp, Artificial Sequence
  3'C_PLP_2
  misc_feature (1)..(1): 5' Phosphate
atgacagcgagaaaaaaaaaaaagtagccgtgactatcgactaaaaaaaaaacgaggatataggc

SEQ ID NO: 21 - DNA, 65 bp, Artificial Sequence; identical to SEQ ID NO: 17
  3'rT_PLP_2
  misc_feature (1)..(1): 5' Phosphate
  misc_feature (65)..(65): RNA

SEQ ID NO: 22 - DNA, 65 bp, Artificial Sequence; identical to SEQ ID NO: 18
  3'rG_PLP_2
  misc_feature (1)..(1): 5' Phosphate
  misc_feature (65)..(65): RNA

SEQ ID NO: 23 - DNA, 65 bp, Artificial Sequence; identical to SEQ ID NO: 19
  3'rA_PLP_2
  misc_feature (1)..(1): 5' Phosphate
  misc_feature (65)..(65): RNA

SEQ ID NO: 24 - DNA, 65 bp, Artificial Sequence; identical to SEQ ID NO: 20
  3'rC_PLP_2
  misc_feature (1)..(1): 5' Phosphate
  misc_feature (65)..(65): RNA

SEQ ID NO: 25 - DNA, 24 bp, Artificial Sequence
  Decorator probe_1
  misc_feature (1)..(1): 5' Phosphate
  misc_feature (21)..(24): 2' O-Me RNA
cctcaatgcacatgtttggctcca

SEQ ID NO: 26 - DNA, 21 bp, Artificial Sequence
  Decorator probe2_2
  misc_feature (1)..(1): 5' Phosphate
  misc_feature (18)..(21): 2' O-Me RNA
agtagccgtgactatcgacta

SEQ ID NO: 27 - RNA, 22 nt, Homo sapiens
ugagguaguagguuguauaguu

SEQ ID NO: 28 - DNA, 59 bp, Artificial Sequence
  let-7a_PLP
ctactacctcaaaaaaaacctcaatgcacatgtttggctccaaaaaaaaactatacaac

SEQ ID NO: 29 - DNA, 79 bp, Artificial Sequence
  iLock_1
cgcgtgtcgttgccctactacctcaaaaaaaaaaacctcaatgcacatgtttggctccaaaaaaaaaaaactatacaac

SEQ ID NO: 30 - DNA, 79 bp, Artificial Sequence; identical to SEQ ID NO: 29
  iLock-3_1
  misc_feature (79)..(79): RNA

SEQ ID NO: 31 - DNA, 79 bp, Artificial Sequence; identical to SEQ ID NO: 29
  iLock-3D_1
  misc_feature (79)..(79): RNA

SEQ ID NO: 32 - DNA, 79 bp, Artificial Sequence; identical to SEQ ID NO: 29
  iLock-3D5_1
  misc_feature (79)..(79): RNA

SEQ ID NO: 33 - DNA, 79 bp, Artificial Sequence; identical to SEQ ID NO: 29
  iLock-3DF_1
  misc_feature (1)..(14): RNA
  misc_feature (79)..(79): RNA

SEQ ID NO: 34 - DNA, 79 bp, Artificial Sequence; identical to SEQ ID NO: 29
  iLock-DF_1
  misc_feature (1)..(14): RNA

SEQ ID NO: 35 - RNA, 25 nt, Artificial Sequence
  benchm_templ_C
ucucgcugucaucccuauauccucg

SEQ ID NO: 36 - RNA, 25 nt, Artificial Sequence
  benchm_templ_A
ucucgcugucauaccuauauccucg

SEQ ID NO: 37 - RNA, 25 nt, Artificial Sequence
  benchm_templ_G
ucucgcugucaugccuauauccucg

SEQ ID NO: 38 - RNA, 25 nt, Artificial Sequence
  benchm_templ_U
ucucgcugucauuccuauauccucg

SEQ ID NO: 39 - DNA, 79 bp, Artificial Sequence
  3'T_iLock_3
tatatccctatattatgacagcgagaaaaaaaaaaaagtagccgtgactatcgactaaaaaaaaaacgaggatataggt

SEQ ID NO: 40 - DNA, 79 bp, Artificial Sequence
  3'G_iLock_3
tatatccctatatgatgacagcgagaaaaaaaaaaaagtagccgtgactatcgactaaaaaaaaaacgaggatataggg

SEQ ID NO: 41 - DNA, 79 bp, Artificial Sequence
  3'A_iLock_3
tatatccctatataatgacagcgagaaaaaaaaaaaagtagccgtgactatcgactaaaaaaaaaacgaggatatagga

SEQ ID NO: 42 - DNA, 79 bp, Artificial Sequence
  3'C_iLock_3
tatatccctatatcatgacagcgagaaaaaaaaaaaagtagccgtgactatcgactaaaaaaaaaacgaggatataggc

SEQ ID NO: 43 - DNA, 79 bp, Artificial Sequence
  3'U_iLock_RNA_3
  misc_feature (13)..(13): RNA
  misc_feature (79)..(79): RNA
tatatccctatatuatgacagcgagaaaaaaaaaaaagtagccgtgactatcgactaaaaaaaaaacgaggatataggu

SEQ ID NO: 44 - DNA, 79 bp, Artificial Sequence; identical to SEQ ID NO: 40
  3'G_iLock_RNA_3
  misc_feature (13)..(13): RNA
  misc_feature (79)..(79): RNA

SEQ ID NO: 45 - DNA, 79 bp, Artificial Sequence; identical to SEQ ID NO: 41
  3'A_iLock _RNA_3
  misc_feature (13)..(13): RNA
  misc_feature (79)..(79): RNA

SEQ ID NO: 46 - DNA, 79 bp, Artificial Sequence; identical to SEQ ID NO: 42
  3'C_iLock _RNA_3
  misc_feature (13)..(13)
  misc_feature (79)..(79)

SEQ ID NO: 47 - DNA, 24 bp, Artificial Sequence
  Decorator probe_1
cctcaatgcacatgtttggctcca

SEQ ID NO: 48 - DNA, 21 bp, Artificial Sequence
  Decorator probe_2
tgcgtctatttagtggagcca

SEQ ID NO: 49 - DNA, 21 bp, Artificial Sequence
  Decorator probe_3
agtagccgtgactatcgacta

SEQ ID NO: 50 - RNA, 22 nt, Homo sapiens
ugagguaguagguuguauaguu

SEQ ID NO: 51 - RNA, 22 nt, Homo sapiens
ugagguaguagauuguauaguu

SEQ ID NO: 52 - RNA, 22 nt, Homo sapiens
ugagguaggagguuguauaguu

SEQ ID NO: 53 - RNA, 22 nt, Homo sapiens
agagguaguagguugcauaguu

SEQ ID NO: 54 - DNA, 69 bp, Artificial Sequence
  let-7a_seqRNA
  misc_feature (14)..(14): RNA
  misc_feature (69)..(69): RNA
aaagatgcgatacactacctcatgcgtctatttagtggagcccgctatcttctttaactatacaaccta

SEQ ID NO: 55 - DNA, 69 bp, Artificial Sequence
  let-7e_seqRNA
  misc_feature (14)..(14): RNA
  misc_feature (69)..(69): RNA
aaaatgtcgttgccctcctacctcatgcgtctatttagtggagccgcctatcttctttaactatacaac

SEQ ID NO: 56 - DNA, 69 bp, Artificial Sequence
  let-7d_seqRNA
  misc_feature (14)..(14): RNA
  misc_feature (69)..(69): RNA
aaaatgtcgttgccctactacctcttgcgtctatttagtggagccatctatcttctttaactatgcaac

SEQ ID NO: 57 - DNA, 69 bp, Artificial Sequence
  let-7f_seqRNA
  misc_feature (14)..(14): RNA
  misc_feature (69)..(69): RNA
aaaatgtcgttgcuctactacctcatgcgtctatttagtggagcctactatcttctttaactatacaau

SEQ ID NO: 58 - DNA, 69 bp, Artificial Sequence; identical to SEQ ID NO: 54
  let-7a_seq

SEQ ID NO: 59 - DNA, 69 bp, Artificial Sequence; identical to SEQ ID NO: 55
  let-7e_seq

SEQ ID NO: 60 - DNA, 69 bp, Artificial Sequence; identical to SEQ ID NO: 56
  let-7d_seq

SEQ ID NO: 61 - DNA, 69 bp, Artificial Sequence
  let-7f_seq
aaaatgtcgttgctctactacctcatgcgtctatttagtggagcctactatcttctttaactatacaat

SEQ ID NO: 62 - DNA, 21 bp, Artificial Sequence
  Decorator probe
  misc_feature (1)..(1): 5' Cy3
tgcgtctatttagtggagcca

SEQ ID NO: 63 - DNA, 21 bp, Artificial Sequence
  anchor primer
  misc_feature (1)..(1): 5' AlexaFluor750
tgcgtctatttagtggagcca

SEQ ID NO: 64 - DNA, 9 bp, Artificial Sequence
  seqlibb1T
  misc_feature (1)..(1): 5' Phosphate
  misc_feature (2)..(9): n is any nucleotide
  misc_feature (9)..(9): 3' FITCb
tnnnnnnnn

SEQ ID NO: 65 - DNA, 9 bp, Artificial Sequence
  seqlibb1G
  misc_feature (1)..(1): 5' Phosphate
  misc_feature (2)..(9): n is any nucleotide
  misc_feature (9)..(9): 3' Cy3b
gnnnnnnnn

SEQ ID NO: 66 - DNA, 9 bp, Artificial Sequence
  seqlibb1A
  misc_feature (1)..(1): 5' Phosphate
  misc_feature (2)..(9): n is any nucleotide
  misc_feature (9)..(9): 3' Cy5b
annnnnnnn

SEQ ID NO: 67 - DNA, 9 bp, Artificial Sequence
  seqlibb1C
  misc_feature (1)..(1): 5' Phosphate
  misc_feature (2)..(9): n is any nucleotide
  misc_feature (9)..(9): 3' TexasRedb
cnnnnnnnn

SEQ ID NO: 68 - DNA, 54 bp, Mus musculus
ggcctgtacactgacttgagaccaataaaagtgcacaccttaccttacacaaac

SEQ ID NO: 69 - DNA, 94 bp, Homo sapiens
tacctgtacactgacttgagaccagttgaataaaagtgcacaccttaaaaatgaaaaaaaaaaaaaaaaaaaaaaaaaaaaaaaaaaaaaaaaa

SEQ ID NO: 70 - DNA, 69 bp, Artificial Sequence
  Mouse PLP
taaggtgtgcaaaaagtagccgtgactatcgactaaaagtagccgtgactatcgactgtttgtgtaagg

SEQ ID NO: 71 - DNA, 68 bp, Artificial Sequence
  Human PLP
taaggtgtgcaagtcggaagtactactctctaaaagtcggaagtactactctctttttttttcatttt

SEQ ID NO: 72 - DNA, 69 bp, Artificial Sequence; identical to SEQ ID NO: 70
  Mouse cPLP
  misc_feature (69)..(69): RNA

SEQ ID NO: 73 - DNA, 68 bp, Artificial Sequence
  Human cPLP
  misc_feature (68)..(68): RNA
taaggtgtgcaagtcggaagtactactctctaaaagtcggaagtactactctctttttttttcatttu

SEQ ID NO: 74 - DNA, 83 bp, Artificial Sequence
  Mouse iLock
tatatccctatatgtaaggtgtgcaaaaagtagccgtgactatcgactaaaagtagccgtgactatcgactgtttgtgtaagg

SEQ ID NO: 75 - DNA, 82 bp, Artificial Sequence
  Human iLock
tatatccctatatttaaggtgtgcaagtcggaagtactactctctaaaagtcggaagtactactctctttttttttcatttt

SEQ ID NO: 76 - DNA, 83 bp, Artificial Sequence; identical to SEQ ID NO: 74
  Mouse ciLock
  misc_feature (14)..(14): RNA
  misc_feature (83)..(83): RNA

SEQ ID NO: 77 - DNA, 82 bp, Artificial Sequence
  Human ciLock
  misc_feature (14)..(14): RNA
  misc_feature (82)..(82): RNA
tatatccctatatutaaggtgtgcaagtcggaagtactactctctaaaagtcggaagtactactctctttttttttcatttu

SEQ ID NO: 78 - RNA, 37 nt, Artificial Sequence
  miR21_BIO
uuuuuuuuuuuuuuuuagcuuaucagacugauguuga

SEQ ID NO: 79 - DNA, 55 bp, Artificial Sequence
  >miR21B2DO_PLP
  misc_feature (1)..(1): 5' Phosphate
ctgataagctagccgaatctaagagtagccgtgactatcgactaaaactacacca

SEQ ID NO: 80 - DNA, 68 bp, Artificial Sequence
  >miR21B2DO_iLock
ccgtcgctgcgttctgataagctaaaaaaaagtagccgtgactatcgactaaaaaaatcaacatcagt

SEQ ID NO: 81 - DNA, 66 bp, Artificial Sequence
  > miR21 B2DO_rPLP
  misc_feature (1)..(1): 5' Phosphate
  misc_feature (1)..(1): Phosphate
  misc_feature (66)..(66): RNA
ctgataagctagccgaatctaagagtagccgtgactatcgactaaaactacaccatcaacatcagu

SEQ ID NO: 82 - DNA, 68 bp, Artificial Sequence
  >miR21B2DO_RiLock
  misc_feature (13)..(13): RNA
  misc_feature (68)..(68): RNA
ccgtcgctgcgtuctgataagctaaaaaaaagtagccgtgactatcgactaaaaaaatcaacatcagu

SEQ ID NO: 83 - DNA, 20 bp, Artificial Sequence
  >B2DO_Cy3
  misc_feature (1)..(1): 5' Cy3
agtagccgtgactatcgact

SEQ ID NO: 84 - DNA, 22 bp, Artificial Sequence
  >antimiR21_FAM
  misc_feature (1)..(1): 5' FAM
tcaacatcagtctgataagcta

SEQ ID NO: 85 - DNA, 99 bp, Homo sapiens
acattttcattatttttattataaggcctgctgaaaatgactgaatataaacttgtggtagttggagctggtggcgtaggcaagagtgccttgacgata

SEQ ID NO: 86 - DNA, 77 bp, Artificial Sequence
  wt KRAS PLP
agctccaactaccacaaagtcgatagtcacggctactcagacgtaacgcgttcagtgatgcccttgcctacgccacc

SEQ ID NO: 87 - RNA, 41 nt, Homo sapiens; identical to SEQ ID NO: 1

SEQ ID NO: 88 - DNA, 77 bp, Artificial Sequence; identical to SEQ ID NO: 86
  chim wt KRAS PLP
  misc_feature (77)..(77): RNA

SEQ ID NO: 89 - DNA, 77 bp, Artificial Sequence; identical to SEQ ID NO: 86
  chim wt KRAS PLP_2
  misc_feature (76)..(77): RNA

SEQ ID NO: 90 - DNA, 80 bp, Artificial Sequence
  mut KRAS PLP
agctccaactaccacaacctcaatgcacatgtttggctcccagacgtaacgcgttcagtgatgcccttgcctacgccact

SEQ ID NO: 91 - DNA, 80 bp, Artificial Sequence
  chim mut KRAS PLP
  misc_feature (80)..(80): RNA
agctccaactaccacaacctcaatgcacatgtttggctcccagacgtaacgcgttcagtgatgcccttgcctacgccacu

SEQ ID NO: 92 - DNA, 15 bp, Artificial Sequence
  RCA primer
catcactgaacgcgt

SEQ ID NO: 93 - DNA, 23 bp, Artificial Sequence
  mut DO-Cy5
cctcaatgcacatgtttggctcc

SEQ ID NO: 94 - DNA, 20 bp, Artificial Sequence
  wt DO-Cy3
agtcgatagtcacggctact

SEQ ID NO: 95 - DNA, 91 bp, Artificial Sequence
  KRAS wt invader chim 3-5
  misc_feature (14)..(14): RNA
  misc_feature (91)..(91): RNA
tatatccctatatcagctccaactaccacaaagtcgatagtcacggctactcagacgtaacgcgttcagtgatgcccttgcctacgccacc

SEQ ID NO: 96 - DNA, 91 bp, Artificial Sequence; identical to SEQ ID NO: 95
  KRAS wt invader chim 3
  misc_feature (14)..(14): RNA
  misc_feature (91)..(91): RNA

SEQ ID NO: 97 - DNA, 94 bp, Artificial Sequence
  KRAS mut invader chim 3-5
  misc_feature (14)..(14): RNA
  misc_feature (94)..(94): RNA
tatatccctatatuagctccaactaccacaacctcaatgcacatgtttggctcccagacgtaacgcgttcagtgatgcccttgcctacgccacu

SEQ ID NO: 98 - DNA, 94 bp, Artificial Sequence
  KRAS mut invader chim 3
  misc_feature (14)..(14): RNA
  misc_feature (94)..(94): RNA
tatatccctatattagctccaactaccacaacctcaatgcacatgtttggctcccagacgtaacgcgttcagtgatgcccttgcctacgccacu

SEQ ID NO: 99 - DNA, 94 bp, Artificial Sequence
  KRAS gapfill invader
tatatctctatatagctccaactaccacaagtagtcgatagtcacggctactcagacgtaacgcgttcagtgatgagtaggcactcttgcctac

SEQ ID NO: 100 - DNA, 19 bp, Artificial Sequence
  invader_splint_chim
  misc_feature (19)..(19): RNA
tatatctctatatgccacc

SEQ ID NO: 101 - DNA, 19 bp, Artificial Sequence
  invader_splint
tatatctctatatgccacc

SEQ ID NO: 102 - DNA, 6 bp, Artificial Sequence
  splint
  misc_feature (6)..(6): RNA
gccacc

SEQ ID NO: 103 - DNA, 6 bp, Artificial Sequence
  splint_chim
gccacc

SEQ ID NO: 104 - DNA, 15 bp, Artificial Sequence
  RCA primer
catcactgaacgcgt

SEQ ID NO: 105 - DNA, 20 bp, Artificial Sequence
  DO-Cy3
agtcgatagtcacggctact

SEQ ID NO: 106 - RNA, 41 nt, Homo sapiens; identical to SEQ ID NO: 1

SEQ ID NO: 107 - DNA, 57 bp, Artificial Sequence
  R_KRAS wt1_1
  misc_feature (20)..(20): RNA
agctccaactaccacaacagacgtaacgcgttcagtgatgcccttgcctacgccacc

SEQ ID NO: 108 - DNA, 57 bp, Artificial Sequence; identical to SEQ ID NO: 107
  R_KRAS wt1_2
  misc_feature (20)..(21): RNA
  misc_feature (29)..(30): RNA

SEQ ID NO: 109 - DNA, 57 bp, Artificial Sequence; identical to SEQ ID NO: 107
  R_KRAS wt1_3
  misc_feature (20)..(22): RNA
  misc_feature (29)..(30): RNA

SEQ ID NO: 110 - DNA, 57 bp, Artificial Sequence; identical to SEQ ID NO: 107
  R_KRAS wt1_4
  misc_feature (20)..(23): RNA
  misc_feature (29)..(30): RNA

SEQ ID NO: 111 - DNA, 57 bp, Artificial Sequence
  R_KRAS wt1_5
  misc_feature (20)..(24): RNA
  misc_feature (29)..(30): RNA
agctccaactaccacaacagacguaacgcgttcagtgatgcccttgcctacgccacc

SEQ ID NO: 112 - DNA, 57 bp, Artificial Sequence; identical to SEQ ID NO: 111
  R_KRAS wt1_7
  misc_feature (20)..(26): RNA
  misc_feature (29)..(30): RNA

SEQ ID NO: 113 - DNA, 57 bp, Artificial Sequence; identical to SEQ ID NO: 111
  R_KRAS wt1_6S
  misc_feature (20)..(21): RNA
  misc_feature (24)..(25): RNA
  misc_feature (28)..(29): RNA

SEQ ID NO: 114 - DNA, 50 bp, Artificial Sequence
  R_KRAS wt1_DNA
agctccaactaccacaaaaaaaaaaaaaaaaaaaacttgcctacgccacc

SEQ ID NO: 115 - DNA, 50 bp, Artificial Sequence; identical to SEQ ID NO: 114
  R_KRAS wt1_RNA
  misc_feature (50)..(50): RNA

SEQ ID NO: 116 - DNA, 22 bp, Artificial Sequence
  Decorator probe [1]
  misc_feature (19)..(22): 2' O-Me RNA
cctcaatgcacatgtttggctc

SEQ ID NO: 117 - DNA, 20 bp, Artificial Sequence
  Decorator probe2 [2]
  misc_feature (17)..(20): 2' O-Me RNA
agtcgatagtcacggctact

SEQ ID NO: 118 - RNA, 41 nt, Homo sapiens; identical to SEQ ID NO: 1

SEQ ID NO: 119 - DNA, 77 bp, Artificial Sequence; identical to SEQ ID NO: 86
  R_KRAS.0

SEQ ID NO: 120 - DNA, 77 bp, Artificial Sequence; identical to SEQ ID NO: 86
  R_KRAS.1G
  misc_feature (40)..(40): RNA

SEQ ID NO: 121 - DNA, 77 bp, Artificial Sequence
  R_KRAS.1C
  misc_feature (40)..(40): RNA
agctccaactaccacaaagtcgatagtcacggctactcacacgtaacgcgttcagtgatgcccttgcctacgccacc

SEQ ID NO: 122 - DNA, 77 bp, Artificial Sequence
  R_KRAS.1A
  misc_feature (40)..(40): RNA
agctccaactaccacaaagtcgatagtcacggctactcaaacgtaacgcgttcagtgatgcccttgcctacgccacc

SEQ ID NO: 123 - DNA, 77 bp, Artificial Sequence
  R_KRAS.1U
  misc_feature (40)..(40): RNA
agctccaactaccacaaagtcgatagtcacggctactcauacgtaacgcgttcagtgatgcccttgcctacgccacc

SEQ ID NO: 124 - DNA, 77 bp, Artificial Sequence
  R_KRAS.2G
  misc_feature (40)..(41): RNA
  misc_feature (49)..(50): RNA
agctccaactaccacaaagtcgatagtcacggctactcaggcgtaacgcgttcagtgatgcccttgcctacgccacc

SEQ ID NO: 125 - DNA, 77 bp, Artificial Sequence
  R_KRAS.2C
  misc_feature (40)..(41): RNA
  misc_feature (49)..(50): RNA
agctccaactaccacaaagtcgatagtcacggctactcacccgtaacgcgttcagtgatgcccttgcctacgccacc

SEQ ID NO: 126 - DNA, 77 bp, Artificial Sequence; identical to SEQ ID NO: 122
  R_KRAS.2A
  misc_feature (40)..(41): RNA
  misc_feature (49)..(50): RNA

SEQ ID NO: 127 - DNA, 77 bp, Artificial Sequence
  R_KRAS.2U
  misc_feature (40)..(41): RNA
  misc_feature (49)..(50): RNA
agctccaactaccacaaagtcgatagtcacggctactcauucgtaacgcgttcagtgatgcccttgcctacgccacc

SEQ ID NO: 128 - DNA, 18 bp, Artificial Sequence
  AluI KRAS RO
cgccaccagctccaacta

SEQ ID NO: 129 - DNA, 53 bp, Artificial Sequence
  PE1
acactctttccctacacgacgctcttccgatctctggtggcgtaggcaagggc

SEQ ID NO: 130 - DNA, 54 bp, Artificial Sequence
  PE2
gtgactggagttcagacgtgtgctcttccgatctctccaactaccacaaagtcg

SEQ ID NO: 131 - DNA, 77 bp, Artificial Sequence
  R_KRAS.3G
  misc_feature (40)..(42): RNA
  misc_feature (49)..(50): RNA
agctccaactaccacaaagtcgatagtcacggctactcagggttaacgcgttcagtgatgcccttgcctacgccacc

SEQ ID NO: 132 - DNA, 77 bp, Artificial Sequence; identical to SEQ ID NO: 125
  R_KRAS.3C
  misc_feature (40)..(42): RNA
  misc_feature (49)..(50): RNA

SEQ ID NO: 133 - DNA, 77 bp, Artificial Sequence
  R_KRAS.3A
  misc_feature (40)..(42): RNA
  misc_feature (49)..(50): RNA
agctccaactaccacaaagtcgatagtcacggctactcaaaagtaacgcgttcagtgatgcccttgcctacgccacc

SEQ ID NO: 134 - DNA, 78 bp, Artificial Sequence
  R_KRAS.3U
  misc_feature (40)..(42): RNA
  misc_feature (49)..(50): RNA
agctccaactaccacaaagtcgatagtcacggctactcauuucgtaacgcgttcagtgatgcccttgcctacgccacc

SEQ ID NO: 135 - DNA, 77 bp, Artificial Sequence
  R_KRAS.5
  misc_feature (40)..(44): RNA
agctccaactaccacaaagtcgatagtcacggctactcagacguaacgcgttcagtgatgcccttgcctacgccacc

SEQ ID NO: 136 - DNA, 77 bp, Artificial Sequence; identical to SEQ ID NO: 135
  R_KRAS.6S
  misc_feature (40)..(41): RNA
  misc_feature (44)..(45): RNA
  misc_feature (48)..(49): RNA

SEQ ID NO: 137 - DNA, 77 bp, Artificial Sequence; identical to SEQ ID NO: 86
  R_KRAS.3
  misc_feature (40)..(42): RNA
  misc_feature (48)..(50): RNA

SEQ ID NO: 138 - DNA, 77 bp, Artificial Sequence; identical to SEQ ID NO: 135
  R_KRAS.3S
  misc_feature (40)..(40)
  misc_feature (42)..(42)
  misc_feature (44)..(44)

SEQ ID NO: 139 - DNA, 77 bp, Artificial Sequence; identical to SEQ ID NO: 86
  R_KRAS.2
  misc_feature (40)..(41): RNA
  misc_feature (49)..(50): RNA

SEQ ID NO: 140 - DNA, 77 bp, Artificial Sequence; identical to SEQ ID NO: 135
  R_KRAS.7
  misc_feature (40)..(46): RNA

SEQ ID NO: 141 - DNA, 20 bp, Artificial Sequence
  Detection probe (seq anchor probe)
  misc_feature (1)..(1): 5' AlexaFluor750
tgcgtctatttagtggagcc

SEQ ID NO: 142 - DNA, 9 bp, Artificial Sequence
  Seq library 1st base-G
  misc_feature (1)..(1): 5' Phosphate
  misc_feature (2)..(4): n is any nucleotide
  misc_feature (9)..(9): 3' Cy3
gnnnctatc

SEQ ID NO: 143 - DNA, 20 bp, Artificial Sequence
  Seq library 1st base-G
  misc_feature (20)..(20): 3' thiophosphate
ggctccactaaatagacgca

SEQ ID NO: 144 - DNA, 9 bp, Artificial Sequence
  Seq library 1st base-A
  misc_feature (1)..(1): 5' Phosphate
  misc_feature (2)..(4): n is any nucleotide
  misc_feature (9)..(9): 3' Cy5
annnctatc

SEQ ID NO: 145 - DNA, 9 bp, Artificial Sequence
  Seq library 1st base-C
  misc_feature (1)..(1): 5' Phosphate
  misc_feature (2)..(4): n is any nucleotide
  misc_feature (9)..(9): 3' TexasRed
cnnnctatc

SEQ ID NO: 146 - DNA, 9 bp, Artificial Sequence
  Seq library 1st base-T
  misc_feature (1)..(1): 5' Phosphate
  misc_feature (2)..(4): n is any nucleotide
  misc_feature (9)..(9): 3' Alexa488
tnnnctatc

SEQ ID NO: 147 - DNA, 9 bp, Artificial Sequence
  Seq library 2nd base-G
  misc_feature (1)..(1): 5' Phosphate
  misc_feature (1)..(1): n is any nucleotide
  misc_feature (3)..(4): n is any nucleotide
  misc_feature (9)..(9): 3' Cy3
ngnnctatc

SEQ ID NO: 148 - DNA, 9 bp, Artificial Sequence
  Seq library 2nd base-A
  misc_feature (1)..(1): 5' Phosphate
  misc_feature (1)..(1): n is any nucleotide
  misc_feature (3)..(4): n is any nucleotide
  misc_feature (9)..(9): 3' Cy5
nannctatc

SEQ ID NO: 149 - DNA, 9 bp, Artificial Sequence
  Seq library 2nd base-C
  misc_feature (1)..(1): 5' Phosphate
  misc_feature (1)..(1): n is any nucleotide
  misc_feature (3)..(4): n is any nucleotide
  misc_feature (9)..(9): 3' TexasRed
ncnnctatc

SEQ ID NO: 150 - DNA, 9 bp, Artificial Sequence
  Seq library 2nd base-T
  misc_feature (1)..(1): 5' Phosphate
  misc_feature (1)..(1): n is any nucleotide
  misc_feature (3)..(4): n is any nucleotide
  misc_feature (9)..(9): 3' Alexa488
ntnnctatc

SEQ ID NO: 151 - DNA, 9 bp, Artificial Sequence
  Seq library 3rd base-G
  misc_feature (1)..(1): 5' Phosphate
  misc_feature (1)..(2): n is any nucleotide
  misc_feature (4)..(4): n is any nucleotide
  misc_feature (9)..(9): 3' Cy3
nngnctatc

SEQ ID NO: 152 - DNA, 9 bp, Artificial Sequence
  Seq library 3rd base-A
  misc_feature (1)..(1): 5' Phosphate
  misc_feature (1)..(2): n is any nucleotide
  misc_feature (4)..(4): n is any nucleotide
  misc_feature (9)..(9): 3' Cy5
nnanctatc

SEQ ID NO: 153 - DNA, 9 bp, Artificial Sequence
  Seq library 3rd base-C
  misc_feature (1)..(1): 5' Phosphate
  misc_feature (1)..(2): n is any nucleotide
  misc_feature (3)..(4): n is any nucleotide
  misc_feature (9)..(9): 3' Cy5
  misc_feature (9)..(9): 3' TexasRed
nncnctatc

SEQ ID NO: 154 - DNA, 9 bp, Artificial Sequence
  Seq library 3rd base-T
  misc_feature (1)..(1): 5' Phosphate
  misc_feature (1)..(1): n is any nucleotide
  misc_feature (2)..(2): n is a, c, g, or t
  misc_feature (3)..(4): n is any nucleotide
  misc_feature (9)..(9): 3' Alexa488
nntnctatc

SEQ ID NO: 155 - DNA, 9 bp, Artificial Sequence
  Seq library 4th base-G
  misc_feature (1)..(1): 5' Phosphate
  misc_feature (1)..(3): n is any nucleotide
  misc_feature (9)..(9): 3' Cy3
nnngctatc

SEQ ID NO: 156 - DNA, 9 bp, Artificial Sequence
  Seq library 4th base-A
  misc_feature (1)..(1): 5' Phosphate
  misc_feature (1)..(3): n is any nucleotide
  misc_feature (9)..(9): 3' Cy5
nnnactatc

SEQ ID NO: 157 - DNA, 9 bp, Artificial Sequence
  Seq library 4th base-C
  misc_feature (1)..(1): 5' Phosphate
  misc_feature (1)..(3): n is any nucleotide
  misc_feature (9)..(9): 3' TexasRed
nnncctatc

SEQ ID NO: 158 - DNA, 9 bp, Artificial Sequence
  Seq library 4th base-T
  misc_feature (1)..(1): 5' Phosphate
  misc_feature (1)..(3): n is any nucleotide
  misc_feature (9)..(9): 3' Alexa488
nnntctatc

SEQ ID NO: 159 - DNA, 95 bp, Artificial Sequence
  Calb2_1119_RNA
  misc_feature (95)..(95): RNA
catcgcagcggagacgacagctgattcctttgactcacattgcgtctatttagtggagccaatgctatcttctttatacagcgaaggaactcatg

SEQ ID NO: 160 - DNA, 95 bp, Artificial Sequence
  Calb2_1328_RNA
  misc_feature (95)..(95): RNA
cacacacgtcaagaacacaactgattcctttgactcacattgcgtctatttagtggagccaatgctatcttctttgaagccaaagagaaaaggaa

SEQ ID NO: 161 - DNA, 95 bp, Artificial Sequence
  Calb2_164_RNA
  misc_feature (95)..(95): RNA
accttcaatgtacccatttcctgattcctttgactcacattgcgtctatttagtggagccaatgctatcttctttaagaagttctctagctcttu

SEQ ID NO: 162 - DNA, 95 bp, Artificial Sequence
  Calb2_500_RNA
  misc_feature (95)..(95): RNA
aggttcatcatagggcctgtctgattcctttgactcacattgcgtctatttagtggagccaatgctatcttcttttgggtgtactcctggagctu

SEQ ID NO: 163 - DNA, 95 bp, Artificial Sequence
  Calb2_937_RNA
  misc_feature (95)..(95): RNA
gtcaagagagtcaggacagcctgattcctttgactcacattgcgtctatttagtggagccaatgctatcttctttggggaggtctgggaaggagu

SEQ ID NO: 164 - DNA, 93 bp, Artificial Sequence
  Calb2_DO3_CCAA_RNA
  misc_feature (93)..(93): RNA
ctcatacagatccttcagctgattcctttgactcacattgcgtctatttagtggagccccaactatcttctttttcatctccttcttgttctu

SEQ ID NO: 165 - DNA, 95 bp, Artificial Sequence
  Chodl_1164_RNA
  misc_feature (95)..(95): RNA
cgggctagtttttgatcttcctgattcctttgactcacattgcgtctatttagtggagccagtactatcttctttatccacagtgtagactgatu

SEQ ID NO: 166 - DNA, 95 bp, Artificial Sequence
  Chodl_1798_RNA
  misc_feature (95)..(95): RNA
aaagcaaagaaacagaacaactgattcctttgactcacattgcgtctatttagtggagccagtactatcttcttttcctaaactttatcgaaccc

SEQ ID NO: 167 - DNA, 95 bp, Artificial Sequence
  Chodl_2071_RNA
  misc_feature (95)..(95): RNA
attctataggcaacatgtgactgattcctttgactcacattgcgtctatttagtggagccagtactatcttctttactctggggagctatttgca

SEQ ID NO: 168 - DNA, 95 bp, Artificial Sequence
  Chodl_2252_RNA
  misc_feature (95)..(95): RNA
gttctgcttagcatcacactctgattcctttgactcacattgcgtctatttagtggagccagtactatcttctttttaatcattaatatcagtgu

SEQ ID NO: 169 - DNA, 95 bp, Artificial Sequence
  Chodl_293_RNA
  misc_feature (95)..(95): RNA
tcctactccctccttcccagctgattcctttgactcacattgcgtctatttagtggagccagtactatcttctttttccttgctttcctgctggg

SEQ ID NO: 170 - DNA, 95 bp, Artificial Sequence
  Chodl_789_RNA
  misc_feature (95)..(95): RNA
gaactgggagctgcttccatctgattcctttgactcacattgcgtctatttagtggagccagtactatcttcttttcatcagtgtaccagtttcg

SEQ ID NO: 171 - DNA, 95 bp, Artificial Sequence
  Chodl_916_RNA
  misc_feature (95)..(95): RNA
tgttgcacctgtcgtcattcctgattcctttgactcacattgcgtctatttagtggagccagtactatcttctttgcagatgtaattgtgcttca

SEQ ID NO: 172 - DNA, 95 bp, Artificial Sequence
  Cort_326_RNA
  misc_feature (95)..(95): RNA
cccgggggtaccccctccgacgtgcttgtggtagcaaatatgcgtctatttagtggagcctgatctatcttctttctttcctggctcttggacag

SEQ ID NO: 173 - DNA, 95 bp, Artificial Sequence
  Cort_529_RNA
  misc_feature (95)..(95): RNA
caaagctgacataagaagaacgtgcttgtggtagcaaatatgcgtctatttagtggagcctgatctatcttctttttctcacagggcaggggagg

SEQ ID NO: 174 - DNA, 95 bp, Artificial Sequence
  Htr3a_1014_GGAC_RNA
  misc_feature (95)..(95): RNA
agtgtgtctgacacgatgatcgtgcttgtggtagcaaatatgcgtctatttagtggagccggacctatcttcttttaccgatggccgttgctggc

SEQ ID NO: 175 - DNA, 95 bp, Artificial Sequence
  Htr3a_1309_GTAA_RNA
  misc_feature (95)..(95): RNA
atggctgcagtggtttcccacgtgcttgtggtagcaaatatgcgtctatttagtggagccgtaactatcttctttaagtcctgaggtcctccaac

SEQ ID NO: 176 - DNA, 95 bp, Artificial Sequence
  Htr3a_1573_TAAC_RNA
  misc_feature (95)..(95): RNA
ccaaatggaccagagagtgacgtgcttgtggtagcaaatatgcgtctatttagtggagcctaacctatcttctttgtgcccactcaagaataatg

SEQ ID NO: 177 - DNA, 95 bp, Artificial Sequence
  Htr3a_1750_TATT_RNA
  misc_feature (95)..(95): RNA
aagtcagagagacagactggcgtgcttgtggtagcaaatatgcgtctatttagtggagcctattctatcttctttgctttaaagccatgataggg

SEQ ID NO: 178 - DNA, 95 bp, Artificial Sequence
  Htr3a_1927_TCGC_RNA
  misc_feature (95)..(95): RNA
gcaagacaatttgcttttctcgtgcttgtggtagcaaatatgcgtctatttagtggagcctcgcctatcttctttcagaagtctcaggcatctau

SEQ ID NO: 179 - DNA, 95 bp, Artificial Sequence
  Htr3a_2045_TGGA_RNA
  misc_feature (95)..(95): RNA
attatcccctgctcccattgcgtgcttgtggtagcaaatatgcgtctatttagtggagcctggactatcttctttttaagatatcatagcatttu

SEQ ID NO: 180 - DNA, 95 bp, Artificial Sequence
  Htr3a_21_AAGT_RNA
  misc_feature (95)..(95): RNA
gtcccaggcagactgcttttcgtgcttgtggtagcaaatatgcgtctatttagtggagccaagtctatcttctttccacccgctgccaacctcau

SEQ ID NO: 181 - DNA, 95 bp, Artificial Sequence
  Htr3a_247_CAGC_RNA
  misc_feature (95)..(95): RNA
gtctgacagccttagtagagcgtgcttgtggtagcaaatatgcgtctatttagtggagcccagcctatcttctttttgtagttagccaggaggtg

SEQ ID NO: 182 - DNA, 95 bp, Artificial Sequence
  Htr3a_424_CGGT_RNA
  misc_feature (95)..(95): RNA
agtccactgcagaaactcatcgtgcttgtggtagcaaatatgcgtctatttagtggagcccggtctatcttctttacattgtcgaagtcctcagg

SEQ ID NO: 183 - DNA, 95 bp, Artificial Sequence
  Htr3a_89_CACT_RNA
  misc_feature (95)..(95): RNA
ctcagagcagccactcaggacgtgcttgtggtagcaaatatgcgtctatttagtggagcccactctatcttctttcttcccagatgtgggagggc

SEQ ID NO: 184 - DNA, 95 bp, Artificial Sequence
  Htr3a_955_GCTC_RNA
  misc_feature (95)..(95): RNA
agagactctctcaccgctgtcgtgcttgtggtagcaaatatgcgtctatttagtggagccgctcctatcttctttagaaggagtgtgatcttgaa

SEQ ID NO: 185 - DNA, 95 bp, Artificial Sequence
  Neurod6_1033_RNA
  misc_feature (95)..(95): RNA
tagaaggattcatatgcactctgattcctttgactcacattgcgtctatttagtggagccttgcctatcttctttactcaggggaggtactttca

SEQ ID NO: 186 - DNA, 95 bp, Artificial Sequence
  Neurod6_108_RNA
  misc_feature (95)..(95): RNA
ctgctagtgacgtcacagggctgattcctttgactcacattgcgtctatttagtggagccttgcctatcttctttagagctggtacccatgccau

SEQ ID NO: 187 - DNA, 95 bp, Artificial Sequence
  Neurod6_1524_RNA
  misc_feature (95)..(95): RNA
tgtgatacagacaagagggactgattcctttgactcacattgcgtctatttagtggagccttgcctatcttctttagagagagagagaatcacag

SEQ ID NO: 188 - DNA, 95 bp, Artificial Sequence
  Neurod6_168_RNA
  misc_feature (95)..(95): RNA
tctcattgatctctaaaaagctgattcctttgactcacattgcgtctatttagtggagccttgcctatcttctttatctgtgtgtatctgcacta

SEQ ID NO: 189 - DNA, 95 bp, Artificial Sequence
  Neurod6_1688_RNA
  misc_feature (95)..(95): RNA
agacattgaagtatgctgtgctgattcctttgactcacattgcgtctatttagtggagccttgcctatcttctttcataactgtacaactgaaau

SEQ ID NO: 190 - DNA, 95 bp, Artificial Sequence
  Neurod6_2041_RNA
  misc_feature (95)..(95): RNA
aacaatacaaaacaagtgctctgattcctttgactcacattgcgtctatttagtggagccttgcctatcttctttacctgtacagaaaaatcctg

SEQ ID NO: 191 - DNA, 95 bp, Artificial Sequence
  Neurod6_228_RNA
  misc_feature (95)..(95): RNA
ttttcaggctgagtgtcgcactgattcctttgactcacattgcgtctatttagtggagccttgcctatcttctttcattttggatcttccaaatc

SEQ ID NO: 192 - DNA, 95 bp, Artificial Sequence
  Neurod6_315_RNA
  misc_feature (95)..(95): RNA
gtagtgttaacatggttcttctgattcctttgactcacattgcgtctatttagtggagccttgcctatcttcttttacgacagactcgtcaaacg

SEQ ID NO: 193 - DNA, 95 bp, Artificial Sequence
  Neurod6_495_RNA
  misc_feature (95)..(95): RNA
tgtcttcttcctcctcttctctgattcctttgactcacattgcgtctatttagtggagccttgcctatcttctttattctcatcttcttcctctc

SEQ ID NO: 194 - DNA, 95 bp, Artificial Sequence
  Neurod6_648_RNA
  misc_feature (95)..(95): RNA
tgtccagagcatcattgaggctgattcctttgactcacattgcgtctatttagtggagccttgcctatcttctttggggaccacttttcgcaaau

SEQ ID NO: 195 - DNA, 95 bp, Artificial Sequence
  Neurod6_714_RNA
  misc_feature (95)..(95): RNA
gtcgtaaagtttctattttgctgattcctttgactcacattgcgtctatttagtggagccttgcctatcttctttccagatgtaatttttggcca

SEQ ID NO: 196 - DNA, 95 bp, Artificial Sequence
  Neurod6_971_RNA
  misc_feature (95)..(95): RNA
cccatgccctgggggagtggctgattcctttgactcacattgcgtctatttagtggagccttgcctatcttctttgacttggaattatcaagagu

SEQ ID NO: 197 - DNA, 92 bp, Artificial Sequence
  Nov_DO2_ATGC_RNA
  misc_feature (92)..(92): RNA
ggagaaagttcatgacactctacgattttaccagtggctgcgtctatttagtggagccatgcctatcttctttgagtcggtttgtctataau

SEQ ID NO: 198 - DNA, 95 bp, Artificial Sequence
  Pcp4_120_RNA
  misc_feature (95)..(95): RNA
tcagaaggcaatgctcagggctgattcctttgactcacattgcgtctatttagtggagccatccctatcttctttgctaggtcccacagaacagc

SEQ ID NO: 199 - DNA, 95 bp, Artificial Sequence
  Pcp4_181_RNA
  misc_feature (95)..(95): RNA
tccggcactttgtctctcacctgattcctttgactcacattgcgtctatttagtggagccatccctatcttctttttgtcttttccgttggtcgc

SEQ ID NO: 200 - DNA, 95 bp, Artificial Sequence
  Pcp4_305_RNA
  misc_feature (95)..(95): RNA
actgagactgaatggccacactgattcctttgactcacattgcgtctatttagtggagccatccctatcttcttttttcttctggaattttctga

SEQ ID NO: 201 - DNA, 95 bp, Artificial Sequence
  Pcp4_386_RNA
  misc_feature (95)..(95): RNA
aacttggtgtcttcaggtggctgattcctttgactcacattgcgtctatttagtggagccatccctatcttctttttcttgatggatggtggttg

SEQ ID NO: 202 - DNA, 95 bp, Artificial Sequence
  Pcp4_472_RNA
  misc_feature (95)..(95): RNA
ttcaggtttgtagcagggtgctgattcctttgactcacattgcgtctatttagtggagccatccctatcttctttatgggtttctcttcatgcau

SEQ ID NO: 203 - DNA, 95 bp, Artificial Sequence
  Pde1a_1081_RNA
  misc_feature (95)..(95): RNA
ttctctgttgagtccgtcagtctacgagtttgcagtcacgtgcgtctatttagtggagccatcgctatcttctttctataagaggaatgacaatu

SEQ ID NO: 204 - DNA, 95 bp, Artificial Sequence
  Pde1a_120_RNA
  misc_feature (95)..(95): RNA
actttggtttttcttcaggctctacgagtttgcagtcacgtgcgtctatttagtggagccatcgctatcttctttagcatggacaatgctgcgaa

SEQ ID NO: 205 - DNA, 95 bp, Artificial Sequence
  Pde1a_1216_RNA
  misc_feature (95)..(95): RNA
tcacacacggagccttttgttctacgagtttgcagtcacgtgcgtctatttagtggagccatcgctatcttctttagtctggggcatagctccca

SEQ ID NO: 206 - DNA, 95 bp, Artificial Sequence
  Pde1a_273_RNA
  misc_feature (95)..(95): RNA
catttaaggcaaatacatcatctacgagtttgcagtcacgtgcgtctatttagtggagccatcgctatcttctttgctatgctccccgcttgctu

SEQ ID NO: 207 - DNA, 95 bp, Artificial Sequence
  Pde1a_334_RNA
  misc_feature (95)..(95): RNA
agatcatatctggtaaagagtctacgagtttgcagtcacgtgcgtctatttagtggagccatcgctatcttctttgaatcttgaagcggttgata

SEQ ID NO: 208 - DNA, 95 bp, Artificial Sequence
  Pde1a_469_RNA
  misc_feature (95)..(95): RNA
atataatgcacagtttgagttctacgagtttgcagtcacgtgcgtctatttagtggagccatcgctatcttcttttgatacctgtatgaagcatu

SEQ ID NO: 209 - DNA, 95 bp, Artificial Sequence
  Pde1a_615_RNA
  misc_feature (95)..(95): RNA
tgtacagaatagcaacgtcctctacgagtttgcagtcacgtgcgtctatttagtggagccatcgctatcttctttctcaagcactgagcggtcgu

SEQ ID NO: 210 - DNA, 95 bp, Artificial Sequence
  Pde1a_759_RNA
  misc_feature (95)..(95): RNA
ctgtcgctaagaccatttcatctacgagtttgcagtcacgtgcgtctatttagtggagccatcgctatcttctttctgaaaatgccctgacatgu

SEQ ID NO: 211 - DNA, 95 bp, Artificial Sequence
  Pde1a_904_RNA
  misc_feature (95)..(95): RNA
ctgtagtgcaacttccaagttctacgagtttgcagtcacgtgcgtctatttagtggagccatcgctatcttctttccattagggccatggtccau

SEQ ID NO: 212 - DNA, 95 bp, Artificial Sequence
  Pde1a_995_RNA
  misc_feature (95)..(95): RNA
cttccgatcacaaagtggagtctacgagtttgcagtcacgtgcgtctatttagtggagccatcgctatcttctttgactgggcaaccattgttga

SEQ ID NO: 213 - DNA, 95 bp, Artificial Sequence
  Penk_1282_RNA
  misc_feature (95)..(95): RNA
caatactgagcttcaagacttctacgattttaccagtggctgcgtctatttagtggagccgtacctatcttctttacaacatagccataagagac

SEQ ID NO: 214 - DNA, 95 bp, Artificial Sequence
  Penk_286_RNA
  misc_feature (95)..(95): RNA
catgggctgtaggagagaagtctacgattttaccagtggctgcgtctatttagtggagccgtacctatcttctttcaaagcctcaggaaccgcgc

SEQ ID NO: 215 - DNA, 95 bp, Artificial Sequence
  Penk_638_RNA
  misc_feature (95)..(95): RNA
gatatagctcgtccatcttctctacgattttaccagtggctgcgtctatttagtggagccgtacctatcttctttttcttcttctggctccatgg

SEQ ID NO: 216 - DNA, 95 bp, Artificial Sequence
  Penk_83_RNA
  misc_feature (95)..(95): RNA
tgcctgggactattctatcttctacgattttaccagtggctgcgtctatttagtggagccgtacctatcttctttgtttcctgctgttctagtga

SEQ ID NO: 217 - DNA, 95 bp, Artificial Sequence
  Penk_882_RNA
  misc_feature (95)..(95): RNA
agttgggggcttcttttgagtctacgattttaccagtggctgcgtctatttagtggagccgtacctatcttctttgctcttttgcttcatcttcc

SEQ ID NO: 218 - DNA, 89 bp, Artificial Sequence
  Plcxd2_DO3_GAAA_RNA
  misc_feature (89)..(89): RNA
gcactcctacacaatgactgattcctttgactcacattgcgtctatttagtggagccgaaactatcttctttgaagatggtgagggtau

SEQ ID NO: 219 - DNA, 90 bp, Artificial Sequence
  Plcxd2_DO3_GGCC_RNA
  misc_feature (90)..(90): RNA
gtggtagaaaatgagaacctgattcctttgactcacattgcgtctatttagtggagccggccctatcttcttttgcttgtagaagggaca

SEQ ID NO: 220 - DNA, 95 bp, Artificial Sequence
  Rorb_2282_RNA
  misc_feature (95)..(95): RNA
tcattcagaattggattccactgattcctttgactcacattgcgtctatttagtggagccaaatctatcttctttataaccaccaaagtgaagtu

SEQ ID NO: 221 - DNA, 95 bp, Artificial Sequence
  Rorb_4479_RNA
  misc_feature (95)..(95): RNA
tcaattttctgccttaagccctgattcctttgactcacattgcgtctatttagtggagccaaatctatcttctttaagaagaaaaagaagttcau

SEQ ID NO: 222 - DNA, 95 bp, Artificial Sequence
  Rorb_536_RNA
  misc_feature (95)..(95): RNA
atgtgaggtcatagataggtctgattcctttgactcacattgcgtctatttagtggagccaaatctatcttctttggtaaacaagttgggtacag

SEQ ID NO: 223 - DNA, 95 bp, Artificial Sequence
  Rorb_6395_RNA
  misc_feature (95)..(95): RNA
gagaaagtgtcacagatttgctgattcctttgactcacattgcgtctatttagtggagccaaatctatcttctttaggtacaattaagagaaagg

SEQ ID NO: 224 - DNA, 95 bp, Artificial Sequence
  Rorb_8435_RNA
  misc_feature (95)..(95): RNA
tagttgttagggagtgctgcctgattcctttgactcacattgcgtctatttagtggagccaaatctatcttctttaagtaatagaaaactctttu

SEQ ID NO: 225 - DNA, 98 bp, Artificial Sequence
  Rorb_DO3_CCGG_RNA
  misc_feature (98)..(98): RNA
agccttttaaagtcatatttggtctgattcctttgactcacattgcgtctatttagtggagccccggctatcttcttaatcggtcatcataaaatacu

SEQ ID NO: 226 - DNA, 87 bp, Artificial Sequence
  Rprm_654_RNA
  misc_feature (87)..(87): RNA
cggtccgtgatggtgcgtgcttgtggtagcaaatatgcgtctatttagtggagccttgtctatcttctttgacaggtttgcgttgcu

SEQ ID NO: 227 - DNA, 74 bp, Artificial Sequence
  Sst_432_AP1SWPLP_RNA
  misc_feature (74)..(74): RNA
taacaggatgtgaatgtcttctacgattttaccagtggcctgactatcttcttttaggacaacaatattaaagc

SEQ ID NO: 228 - DNA, 95 bp, Artificial Sequence
  Synpr_1071_RNA
  misc_feature (95)..(95): RNA
catactagagactttaagcttctacgattttaccagtggctgcgtctatttagtggagccattactatcttctttaaggtaatctatgcacatta

SEQ ID NO: 229 - DNA, 95 bp, Artificial Sequence
  Synpr_1643_RNA
  misc_feature (95)..(95): RNA
cctctctggatgcaaagaaatctacgattttaccagtggctgcgtctatttagtggagccattactatcttctttaactatggtgtctaaatctg

SEQ ID NO: 230 - DNA, 95 bp, Artificial Sequence
  Synpr_260_RNA
  misc_feature (95)..(95): RNA
atgtacacgaccgtggcagctctacgattttaccagtggctgcgtctatttagtggagccattactatcttctttggtacttgttctggaagaaa

SEQ ID NO: 231 - DNA, 95 bp, Artificial Sequence
  Synpr_591_RNA
  misc_feature (95)..(95): RNA
aaggtatctctgtccagaggtctacgattttaccagtggctgcgtctatttagtggagccattactatcttcttttgcttctccatggggtctga

SEQ ID NO: 232 - DNA, 98 bp, Artificial Sequence
  Synpr_DO2_ATTA_RNA
  misc_feature (98)..(98): RNA
cttaaaaattcttctgctactggtctacgattttaccagtggctgcgtctatttagtggagccattactatcttcttcattaataattgattgaaacu

SEQ ID NO: 233 - DNA, 95 bp, Artificial Sequence
  Yjefn3_138_RNA
  misc_feature (95)..(95): RNA
cactagcgtgcccacatagtcgtgcttgtggtagcaaatatgcgtctatttagtggagcctttactatcttctttggccttggtcacagccaccg

SEQ ID NO: 234 - DNA, 95 bp, Artificial Sequence
  Yjefn3_344_RNA
  misc_feature (95)..(95): RNA
cttctcgcactgcgtggtcacgtgcttgtggtagcaaatatgcgtctatttagtggagcctttactatcttctttgacaggaaggggatgtccau

SEQ ID NO: 235 - DNA, 95 bp, Artificial Sequence
  Yjefn3_686_RNA
  misc_feature (95)..(95): RNA
aaactttcggcggacgtcatcgtgcttgtggtagcaaatatgcgtctatttagtggagcctttactatcttcttttattttggcaggtgcaggcc

SEQ ID NO: 236 - DNA, 95 bp, Artificial Sequence
  Bgn_412_RNA
  misc_feature (95)..(95): RNA
gggcacagtcttcagacccatctacgattttaccagtggctgcgtctatttagtggagccctatctatcttctttgtgtcaggtgagatctcctu

SEQ ID NO: 237 - DNA, 95 bp, Artificial Sequence
  Bgn_851_RNA
  misc_feature (95)..(95): RNA
tcagggtctcagggagatcttctacgattttaccagtggctgcgtctatttagtggagccctatctatcttctttgtggtccaggtgaagttcgu

SEQ ID NO: 238 - DNA, 95 bp, Artificial Sequence
  Bgn_1194_RNA
  misc_feature (95)..(95): RNA
tcccagtagggcacagggtttctacgattttaccagtggctgcgtctatttagtggagccctatctatcttctttggaaggtggcaggctgcacu

SEQ ID NO: 239 - DNA, 95 bp, Artificial Sequence
  Bgn_1577_RNA
  misc_feature (95)..(95): RNA
aacaatggcggtggcagtgttctacgattttaccagtggctgcgtctatttagtggagccctatctatcttctttaggaacacatgcctggatgg

SEQ ID NO: 240 - DNA, 95 bp, Artificial Sequence
  Bgn_2309_RNA
  misc_feature (95)..(95): RNA
tcagggacccaggggtgaggtctacgattttaccagtggctgcgtctatttagtggagccctatctatcttctttgaccatcacctcctaccaca

SEQ ID NO: 241 - DNA, 95 bp, Artificial Sequence
  Apq4_879_RNA
  misc_feature (95)..(95): RNA
cttaaggcgacgtttgagctctgattcctttgactcacattgcgtctatttagtggagcccattctatcttctttgcggctttgctgaaggcttc

SEQ ID NO: 242 - DNA, 95 bp, Artificial Sequence
  Apq4_2186_RNA
  misc_feature (95)..(95): RNA
aattacactcacaatgccgactgattcctttgactcacattgcgtctatttagtggagcccattctatcttcttttaattcacacaaatgggtau

SEQ ID NO: 243 - DNA, 95 bp, Artificial Sequence
  Apq4_3100_RNA
  misc_feature (95)..(95): RNA
cactggaaatgactgttaaactgattcctttgactcacattgcgtctatttagtggagcccattctatcttcttttgtaccatactgaatgctgu

SEQ ID NO: 244 - DNA, 95 bp, Artificial Sequence
  Apq4_3673_RNA
  misc_feature (95)..(95): RNA
cggtgtatctgtcagtagctctgattcctttgactcacattgcgtctatttagtggagcccattctatcttcttttttcctctctgatctctgtg

SEQ ID NO: 245 - DNA, 95 bp, Artificial Sequence
  Apq4_4344_RNA
  misc_feature (95)..(95): RNA
acagaggcagtgtctctgtgctgattcctttgactcacattgcgtctatttagtggagcccattctatcttctttgctctctggcttcaattgtc

SEQ ID NO: 246 - DNA, 95 bp, Artificial Sequence
  Pdgfra_296_RNA
  misc_feature (95)..(95): RNA
tgggaggatagagggtaatatctacgagtttgcagtcacgtgcgtctatttagtggagcctgtcctatcttctttacaatcttctcattctcgtu

SEQ ID NO: 247 - DNA, 95 bp, Artificial Sequence
  Pdgfra_646_RNA
  misc_feature (95)..(95): RNA
ggtatgatggcagagtcatctctacgagtttgcagtcacgtgcgtctatttagtggagcctgtcctatcttctttccggatctgtggtgcggcaa

SEQ ID NO: 248 - DNA, 95 bp, Artificial Sequence
  Pdgfra_832_RNA
  misc_feature (95)..(95): RNA
gttgctttcaaggcataaactctacgagtttgcagtcacgtgcgtctatttagtggagcctgtcctatcttcttttctccagattcagttctgac

SEQ ID NO: 249 - DNA, 95 bp, Artificial Sequence
  Pdgfra_1227_RNA
  misc_feature (95)..(95): RNA
ggtaggcctgcacctccacctctacgagtttgcagtcacgtgcgtctatttagtggagcctgtcctatcttctttccacgatatcctgggcgtcg

SEQ ID NO: 250 - DNA, 95 bp, Artificial Sequence
  Pdgfra_1544_RNA
  misc_feature (95)..(95): RNA
catccagtcgatttctggaatctacgagtttgcagtcacgtgcgtctatttagtggagcctgtcctatcttctttttcttaatatgcttgcagau

SEQ ID NO: 251 - DNA, 57 bp, Artificial Sequence
  fwd_index1
aatgatacggcgaccaccgagatctacacaggctataacactctttccctacacgac

SEQ ID NO: 252 - DNA, 57 bp, Artificial Sequence
  fwd_index2
aatgatacggcgaccaccgagatctacacgcctctatacactctttccctacacgac

SEQ ID NO: 253 - DNA, 57 bp, Artificial Sequence
  fwd_index3
aatgatacggcgaccaccgagatctacacaggataggacactctttccctacacgac

SEQ ID NO: 254 - DNA, 57 bp, Artificial Sequence
  fwd_index4
aatgatacggcgaccaccgagatctacactcagagccacactctttccctacacgac

SEQ ID NO: 255 - DNA, 57 bp, Artificial Sequence
  fwd_index5
aatgatacggcgaccaccgagatctacaccttcgcctacactctttccctacacgac

SEQ ID NO: 256 - DNA, 57 bp, Artificial Sequence
  fwd_index6
aatgatacggcgaccaccgagatctacactaagattaacactctttccctacacgac

SEQ ID NO: 257 - DNA, 57 bp, Artificial Sequence
  fwd_index7
aatgatacggcgaccaccgagatctacacacgtcctgacactctttccctacacgac

SEQ ID NO: 258 - DNA, 57 bp, Artificial Sequence
  fwd_index8
aatgatacggcgaccaccgagatctacacgtcagtacacactctttccctacacgac

SEQ ID NO: 259 - DNA, 53 bp, Artificial Sequence
  rev_index1
caagcagaagacggcatacgagatcgagtaatgtgactggagttcagacgtgt

SEQ ID NO: 260 - DNA, 53 bp, Artificial Sequence
  rev_index2
caagcagaagacggcatacgagattctccggagtgactggagttcagacgtgt

SEQ ID NO: 261 - DNA, 53 bp, Artificial Sequence
  rev_index3
caagcagaagacggcatacgagataatgagcggtgactggagttcagacgtgt

SEQ ID NO: 262 - DNA, 20 bp, Artificial Sequence
  P5primer
aatgatacggcgaccaccga

SEQ ID NO: 263 - DNA, 21 bp, Artificial Sequence
  P7primer
caagcagaagacggcatacga

SEQ ID NO: 264 - DNA, 77 bp, Artificial Sequence
  R_KRAS.D3
  misc_feature (24)..(24): RNA
  misc_feature (40)..(40): RNA
  misc_feature (56)..(56): RNA
agctccaactaccacaaagtcgauagtcacggctactcagacgtaacgcgttcagugatgcccttgcctacgccacc

SEQ ID NO: 265 - DNA, 77 bp, Artificial Sequence; identical to SEQ ID NO: 264
  R_KRAS.D8
  misc_feature (18)..(18): RNA
  misc_feature (24)..(24): RNA
  misc_feature (30)..(30): RNA
  misc_feature (36)..(36): RNA
  misc_feature (42)..(42): RNA
  misc_feature (49)..(49): RNA
  misc_feature (56)..(56): RNA
  misc_feature (62)..(62): RNA

SEQ ID NO: 266 - protein, 575 aa, Bacteriophage phi-29 [sequence omitted]

SEQ ID NO: 267 - DNA, 77 bp, Artificial Sequence; identical to SEQ ID NO: 124
  R_KRAS.2G
  misc_feature (40)..(41): RNA

SEQ ID NO: 268 - DNA, 77 bp, Artificial Sequence; identical to SEQ ID NO: 125
  R_KRAS.2C
  misc_feature (40)..(41): RNA

SEQ ID NO: 269 - DNA, 77 bp, Artificial Sequence; identical to SEQ ID NO: 122
  R_KRAS.2A
  misc_feature (40)..(41): RNA

SEQ ID NO: 270 - DNA, 77 bp, Artificial Sequence; identical to SEQ ID NO: 127
  R_KRAS.2U
  misc_feature (40)..(41): RNA

SEQ ID NO: 271 - DNA, 77 bp, Artificial Sequence; identical to SEQ ID NO: 131
  R_KRAS.3G
  misc_feature (40)..(42): RNA

SEQ ID NO: 272 - DNA, 77 bp, Artificial Sequence; identical to SEQ ID NO: 125
  R_KRAS.3C
  misc_feature (40)..(42): RNA

SEQ ID NO: 273 - DNA, 77 bp, Artificial Sequence; identical to SEQ ID NO: 133
  R_KRAS.3A
  misc_feature (40)..(42): RNA

SEQ ID NO: 274 - DNA, 78 bp, Artificial Sequence; identical to SEQ ID NO: 134
  R_KRAS.3U
  misc_feature (40)..(42): RNA

SEQ ID NO: 275 - DNA, 77 bp, Artificial Sequence; identical to SEQ ID NO: 86
  R_KRAS.3
  misc_feature (40)..(42): RNA

SEQ ID NO: 276 - DNA, 77 bp, Artificial Sequence; identical to SEQ ID NO: 86
  R_KRAS.2
  misc_feature (40)..(41): RNA

SEQ ID NO: 277 - DNA, 57 bp, Artificial Sequence; identical to SEQ ID NO: 107
  R_KRAS wt1_2
  misc_feature (20)..(21): RNA

SEQ ID NO: 278 - DNA, 57 bp, Artificial Sequence; identical to SEQ ID NO: 107
  R_KRAS wt1_3
  misc_feature (20)..(22): RNA

SEQ ID NO: 279 - DNA, 57 bp, Artificial Sequence; identical to SEQ ID NO: 107
  R_KRAS wt1_4
  misc_feature (20)..(23): RNA

SEQ ID NO: 280 - DNA, 57 bp, Artificial Sequence; identical to SEQ ID NO: 111
  R_KRAS wt1_5
  misc_feature (20)..(24): RNA

SEQ ID NO: 281 - DNA, 57 bp, Artificial Sequence; identical to SEQ ID NO: 111
  R_KRAS wt1_7
  misc_feature (20)..(26): RNA